European Patent Application EP 4 556 558 A1, published May 21, 2025. Title: Mutant microorganism of Corynebacterium genus producing L-glutamic acid and method for producing L-glutamic acid using the same. Applicant: DAESANG CORPORATION. The sequence listing filed with the application follows.

SEQUENCE LISTING (9 sequences)

SEQ ID NO: 1 - DNA, 1086 bp, synthetic construct
  source 1..1086: mol_type = other DNA
atggcagtcatggcatatcaaccagcagacaatcgctatgacgacatgatctaccgcagggtgggaaattctgggctgaagcttccggcaatttcgcttgggctgtggcacaacttcggtgatgacaagccgctttcaacgcagcgcagcattattcaccgcgcgtttgataggggagtcacccacttcgatttggctaataactatggacctccagcaggttccgcggagacaaactttggcaggattttgcgtgaggatctcaaaaaccaccgcgatgagttgatcatttcttccaaggcgggttgggatatgtggcctggaccttatggttttggtggttcccgaaagtatctagtgagttcccttgatcagtccctgactcgcctcggcttggattacgtggatattttctaccaccaccgcccggacccagacactcctttggaagaaaccatgtacgcattgcgtgacattgttgcgtctggaaaggctctttacgtgggtatttcttcctacggtccagagctcacagcggaggctgctgagttcatggcggaggagggctgcccgcttctgattcatcagccaagttattccatcattaatcgttgggtggaggaaccgggcgatgacggtgagaacttgttgcagtcagctgccaacaatggtcttggcgtcattgctttctcaccacttgcgcagggcctgctcacggacaaatatctcgatggaattccagagggttcccgcgccagccagggtaagtccctgtctgagggcatgttgaacgtgaacaatattgatatggtccgcaagctcaatgacatcgctcaggaacgcgggcagtcacttgcgcagatggcgcttgcatgggtgctgcgcgagcaaggagagtacggcgcggataccgtgaccagtgcattgattggtgcttcgtcagttgagcagctggacaacaaccttgattcactcaacaacttggagttttctgacgccgagttggaggcgatcgatgagatttcccacgacgctggcatcaacatttgggcgaaggccaccgattctaaaacccgcgaaaactaa

SEQ ID NO: 2 - protein, 361 aa, synthetic construct
MAVMAYQPADNRYDDMIYRRVGNSGLKLPAISLGLWHNFGDDKPLSTQRSIIHRAFDRGVTHFDLANNYGPPAGSAETNFGRILREDLKNHRDELIISSKAGWDMWPGPYGFGGSRKYLVSSLDQSLTRLGLDYVDIFYHHRPDPDTPLEETMYALRDIVASGKALYVGISSYGPELTAEAAEFMAEEGCPLLIHQPSYSIINRWVEEPGDDGENLLQSAANNGLGVIAFSPLAQGLLTDKYLDGIPEGSRASQGKSLSEGMLNVNNIDMVRKLNDIAQERGQSLAQMALAWVLREQGEYGADTVTSALIGASSVEQLDNNLDSLNNLEFSDAELEAIDEISHDAGINIWAKATDSKTREN

SEQ ID NO: 3 - DNA, 1086 bp, Corynebacterium sp.
  source 1..1086: mol_type = genomic DNA
atggcagtcatggcatatcaaccagcagacaatcgctatgacgacatgatctaccgcagggtgggaaattctgggctgaagcttccggcaatttcgcttgggctgtggcacaacttcggtgatgacaagccgctttcaacgcagcgcagcattattcaccgcgcgtttgataggggagtcacccacttcgatttggctaataactatggacctccagcaggttccgcggagacaaactttggcaggattttgcgtgaggatctcaaaaaccaccgcgatgagttgatcatttcttccaaggcgggttgggatatgtggcctggaccttatggttttggtggttcccgaaagtatctagtgagttcccttgatcagtccctgactcgcctcggcttggattacgtggatattttctaccaccaccgcccggacccagacactcctttggaagaaaccatgtacgcattgcgtgacattgttgcgtctggaaaggctctttacgtgggtatttcttcctacggtccagagctcacagcggaggctgctgagttcatggcggaggagggctgcccgcttctgattcatcagccaagttattccatcattaatcgttgggtggaggaaccgggcgatgacggtgagaacttgttgcagtcagctgccaacaatggtcttggcgtcattgctttctcaccacttgcgcagggcctgctcacggacaaatatctcgatggaattccagagggttcccgcgccagccagggtaagtccctgtctgagggcatgttgaacgtgaacaatattgatatggtccgcaagctcaatgacatcgctcaggaacgcgggcagtcacttgcgcagatggcgcttgcatgggtgctgcgcgagcaaggagagtacggcgcggataccgtgaccagtgcattgattggtgcttcgtcagttgagcagctggacaacagccttgattcactcaacaacttggagttttctgacgccgagttggaggcgatcgatgagatttcccacgacgctggcatcaacatttgggcgaaggccaccgattctaaaacccgcgaaaactaa

SEQ ID NO: 4 - protein, 361 aa, Corynebacterium sp.
MAVMAYQPADNRYDDMIYRRVGNSGLKLPAISLGLWHNFGDDKPLSTQRSIIHRAFDRGVTHFDLANNYGPPAGSAETNFGRILREDLKNHRDELIISSKAGWDMWPGPYGFGGSRKYLVSSLDQSLTRLGLDYVDIFYHHRPDPDTPLEETMYALRDIVASGKALYVGISSYGPELTAEAAEFMAEEGCPLLIHQPSYSIINRWVEEPGDDGENLLQSAANNGLGVIAFSPLAQGLLTDKYLDGIPEGSRASQGKSLSEGMLNVNNIDMVRKLNDIAQERGQSLAQMALAWVLREQGEYGADTVTSALIGASSVEQLDNSLDSLNNLEFSDAELEAIDEISHDAGINIWAKATDSKTREN

SEQ ID NO: 5 - DNA, 5719 bp, synthetic construct
  source 1..5719: mol_type = other DNA
tgccgcaagcactcagggcgcaagggctgctaaaggaagcggaacacgtagaaagccagtccgcagaaacggtgctgaccccggatgaatgtcagctactgggctatctggacaagggaaaacgcaagcgcaaagagaaagcaggtagcttgcagtgggcttacatggcgatagctagactgggcggttttatggacagcaagcgaaccggaattgccagctggggcgccctctggtaaggttgggaagccctgcaaagtaaactggatggctttcttgccgccaaggatctgatggcgcaggggatcaagatctgatcaagagacaggatgaggatcgtttcgcatgattgaacaagatggattgcacgcaggttctccggccgcttgggtggagaggctattcggctatgactgggcacaacagacaatcggctgctctgatgccgccgtgttccggctgtcagcgcaggggcgcccggttctttttgtcaagaccgacctgtccggtgccctgaatgaactccaagacgaggcagcgcggctatcgtggctggccacgacgggcgttccttgcgcagctgtgctcgacgttgtcactgaagcgggaagggactggctgctattgggcgaagtgccggggcaggatctcctgtcatctcaccttgctcctgccgagaaagtatccatcatggctgatgcaatgcggcggctgcatacgcttgatccggctacctgcccattcgaccaccaagcgaaacatcgcatcgagcgagcacgtactcggatggaagccggtcttgtcgatcaggatgatctggacgaagagcatcaggggctcgcgccagccgaactgttcgccaggctcaaggcgcggatgcccgacggcgaggatctcgtcgtgacccatggcgatgcctgcttgccgaatatcatggtggaaaatggccgcttttctggattcatcgactgtggccggctgggtgtggcggaccgctatcaggacatagcgttggctacccgtgatattgctgaagagcttggcggcgaatgggctgaccgcttcctcgtgctttacggtatcgccgctcccgattcgcagcgcatcgccttctatcgccttcttgacgagttcttctgagcgggactctggggttcgctagaggatcgatcctttttaacccatcacatatacctgccgttcactattatttagtgaaatgagatattatgatattttctgaattgtgattaaaaaggcaactttatgcccatgcaacagaaactataaaaaatacagagaatgaaaagaaacagatagattttttagttctttaggcccgtagtctgcaaatccttttatgattttctatcaaacaaaagaggaaaatagaccagttgcaatccaaacgagagtctaatagaatgaggtcgaaaagtaaatcgcgcgggtttgttactgataaagcaggcaagacctaaaatgtgtaaagggcaaagtgtatactttggcgtcaccccttacatattttaggtctttttttattgtgcgtaactaacttgccatcttcaaacaggagggctggaagaagcagaccgctaacacagtacataaaaaaggagacatgaacgatgaacatcaaaaagtttgcaaaacaagcaacagtattaacctttactaccgcactgctggcaggaggcgcaactcaagcgtttgcgaaagaaacgaaccaaaagccatataaggaaacatacggcatttcccatattacacgccatgatatgctgcaaatccctgaacagcaaaaaaatgaaaaatatcaagtttctgaatttgattcgtccacaattaaaaatatctcttctgcaaaaggcctggacgtttgggacagctggccattacaaaacgctgacggcactgtcgcaaactatcacggctaccacatcgtctttgcattagccggagatcctaaaaatgcggatgacacatcgatttacatgttctatcaaaaagtcggcgaaacttctattgacagctggaaaaacgctggccgcgtctttaaagacagcgacaaattcgatgcaaatgattctatcctaaaagaccaaacacaagaatggtcaggttcagccacatttacatctgacggaaaaatccgtttattctacactgatttctccggtaaacattacggcaaacaaacactgacaactgcacaagttaacgtatcagcatcagacagctctttgaacatcaacggtgtagaggattataaatcaatctttgacggtgacggaaaaacgtatcaaaatgtacagcagttcatcgatgaaggcaactacagctcaggcgacaaccatacgctgagagatcctcactacgtagaagataaaggccacaaatacttagtatttgaagcaaacactggaactgaagatggctaccaaggcgaagaatctttatttaacaaagcatactatggcaaaagcacatcattcttccgtcaagaaagtcaaaaacttctgcaaagcgataaaaaacgcacggctgagttagcaaacggcgctctcggtatgattgagctaaacgatgattacacactgaaaaaagtgatgaaaccgctgattgcatctaacacagtaacagatgaaattgaacgcgcgaacgtctttaaaatgaacggcaaatggtacctgttcactgactcccgcggatcaaaaatgacgattgacggcattacgtctaacgatatttacatgcttggttatgtttctaattctttaactggcccatacaagccgctgaacaaaactggccttgtgttaaaaatggatcttgatcctaacgatgtaacctttacttactcacacttcgctgtacctcaagcgaaaggaaacaatgtcgtgattacaagctatatgacaaacagaggattctacgcagacaaacaatcaacgtttgcgccgagcttcctgctgaacatcaaaggcaagaaaacatctgttgtcaaagacagcatccttgaacaaggacaattaacagttaacaaataaaaacgcaaaagaaaatgccgatgggtaccgagcgaaatgaccgaccaagcgacgcccaacctgccatcacgagatttcgattccaccgccgccttctatgaaaggttgggcttcggaatcgttttccgggacgccctcgcggacgtgctcatagtccacgacgcccgtgattttgtagccctggccgacggccagcaggtaggccgacaggctcatgccggccgccgccgccttttcctcaatcgctcttcgttcgtctggaaggcagtacaccttgataggtgggctgcccttcctggttggcttggtttcatcagccatccgcttgccctcatctgttacgccggcggtagccggccagcctcgcagagcaggattcccgttgagcaccgccaggtgcgaataagggacagtgaagaaggaacacccgctcgcgggtgggcctacttcacctatcctgcccggctgacgccgttggatacaccaaggaaagtctacacgaaccctttggcaaaatcctgtatatcgtgcgaaaaaggatggatataccgaaaaaatcgctataatgaccccgaagcagggttatgcagcggaaaagcgctgcttccctgctgttttgtggaatatctaccgactggaaacaggcaaatgcaggaaattactgaactgaggggacaggcgagagacgatgccaaagagctcctgaaaatctcgataactcaaaaaatacgcccggtagtgatcttatttcattatggtgaaagttggaacctcttacgtgccgatcaacgtctcattttcgccaaaagttggcccagggcttcccggtatcaacagggacaccaggatttatttattctgcgaagtgatcttccgtcacaggtatttattcggcgcaaagtgcgtcgggtgatgctgccaacttactgatttagtgtatgatggtgtttttgaggtgctccagtggcttctgtttctatcagctcctgaaaatctcgataactcaaaaaatacgcccggtagtgatcttatttcattatggtgaaagttggaacctcttacgtgccgatcaacgtctcattttcgccaaaagttggcccagggcttcccggtatcaacagggacaccaggatttatttattctgcgaagtgatcttccgtcacaggtatttattcggcgcaaagtgcgtcgggtgatgctgccaacttactgatttagtgtatgatggtgtttttgaggtgctccagtggcttctgtttctatcagggctggatgatcctccagcgcggggatctcatgctggagttcttcgcccaccccaaaaggatctaggtgaagatcctttttgataatctcatgaccaaaatcccttaacgtgagttttcgttccactgagcgtcagaccccgtagaaaagatcaaaggatcttcttgagatcctttttttctgcgcgtaatctgctgcttgcaaacaaaaaaaccaccgctaccagcggtggtttgtttgccggatcaagagctaccaactctttttccgaaggtaactggcttcagcagagcgcagataccaaatactgttcttctagtgtagccgtagttaggccaccacttcaagaactctgtagcaccgcctacatacctcgctctgctaatcctgttaccagtggctgctgccagtggcgataagtcgtgtcttaccgggttggactcaagacgatagttaccggataaggcgcagcggtcgggctgaacggggggttcgtgcacacagcccagcttggagcgaacgacctacaccgaactgagatacctacagcgtgagctatgagaaagcgccacgcttcccgaagggagaaaggcggacaggtatccggtaagcggcagggtcggaacaggagagcgcacgagggagcttccagggggaaacgcctggtatctttatagtcctgtcgggtttcgccacctctgacttgagcgtcgatttttgtgatgctcgtcaggggggcggagcctatggaaaaacgccagcaacgcggcctttttacggttcctggccttttgctggccttttgctcacatgttctttcctgcgttatcccctgattctgtggataaccgtattaccgcctttgagtgagctgataccgctcgccgcagccgaacgaccgagcgcagcgagtcagtgagcgaggaagcggaagagcgcccaatacgcaaaccgcctctccccgcgcgttggccgattcattaatgcagctggcacgacaggtttcccgactggaaagcgggcagtgagcgcaacgcaattaatgtgagttagctcactcattaggcaccccaggctttacactttatgcttccggctcgtatgttgtgtggaattgtgagcggataacaatttcacacaggaaacagctatgacatgattacgccaagcttgcatgcctgcaggtcgactctagaggatccccgggtaccgagctcgaattcactggccgtcgttttacaacgtcgtgactgggaaaaccctggcgttacccaacttaatcgccttgcagcacatccccctttcgccagctggcgtaatagcgaagaggcccgcaccgatcgcccttcccaacagttgcgcagcctgaatggcgaatggcgataagctagcttcacgc

SEQ ID NO: 6 - DNA, 18 bp, synthetic construct
  source 1..18: mol_type = other DNA
acctccagcaggttccgc

SEQ ID NO: 7 - DNA, 24 bp, synthetic construct
  source 1..24: mol_type = other DNA
agtgaatcaaggttgttgtccagc

SEQ ID NO: 8 - DNA, 24 bp, synthetic construct
  source 1..24: mol_type = other DNA
gctggacaacaaccttgattcact

SEQ ID NO: 9 - DNA, 23 bp, synthetic construct
  source 1..23: mol_type = other DNA
ctgacgtctttttgttcatcgcc